European Patent Application EP 4 545 628 A1, published April 30, 2025. Title: LIMOSILACTOBACILLUS FERMENTUM MSJK0025 FROM BREAST MILK FOR ADJUSTING GUT MICROBIOTA AND APPLICATION THEREOF. Applicant: ZHEJIANG MINSHENG HEALTHCARE CO., LTD. Application WO PCT/CN2023/143049, filed December 29, 2023. The sequence listing filed with the application follows.

SEQUENCE LISTING (1 sequence)

SEQ ID NO: 1 - RNA, 1004 nt, Limosilactobacillus fermentum
  source 1..1004: mol_type = rRNA
aattgattgatggtgcttgcacctgattgattttggtcgccaacgagtggcggacgggtgagtaacacgtaggtaacctgcccagaagcgggggacaacatttggaaacagatgctaataccgcataacaacgttgttcgcatgaacaacgcttaaaagatggcatatcgctatcacttctggatggacctgcggtgcattagcttgttggtggggtaacggcctaccaaggcgatgatgcatagccgagttgagagactgatcggccacaatgggactgagacacggcccatactcctacgggaggcagcagtagggaatcttccacaatgggcgcaagcctgatggagcaacaccgcgtgagtgaagaagggtttcggctcgtaaagctctgttgtaaaagaagaacacgtatgagagtaactgttcatacgttgacggtatttaaccagaaagtcacggctaactacgtgccagcagccgcggtaatacgtaggtggcaagcgttatccggatttattgggcgtaaagagagtgcaggcggttttctaagtvtgatgtgaaagccttcggcttaaccggagaagtgcatcggaaactggataacttgagtgcagaagagggtagtggaactccatgtgtagcggtggaatgcgtagatatatggaagaacaccagtggcgaaggcggctacctggtctgcaactgacgctgagactcgaaagcatgggtagcgaacaggattagataccctggtagtccatgccgtaaacgatgagtgctaggtgttggagggtttccgcccttcagtgccggagctaacgcattaagcactccgcctggggagtacgaccgcaaggttgaaactcaaaggaattgacgggggcccgcacaagcggtggagcatgtggtttaattcgaagctacgcgaagaaccttaccaggtcttgacatcttgcgccaaccctagagatagggcgtttccttcgggaacgcaatgacag